European Patent Application EP 4 428 153 A1, published September 11, 2024. Title: 结合GPRC5D的抗体及其用途. Applicant: 正大天晴药业集团股份有限公司. The sequence listing filed with the application follows.

SEQUENCE LISTING (71 sequences)

SEQ ID NO: 1 - protein, 10 aa, Mus musculus
GYTFTNYVMH

SEQ ID NO: 2 - protein, 17 aa, Mus musculus
YFNPYNDGTNYNEKFKG

SEQ ID NO: 3 - protein, 9 aa, Mus musculus
GGVRRYFDV

SEQ ID NO: 4 - protein, 11 aa, Mus musculus
RASQDIGSNLN

SEQ ID NO: 5 - protein, 7 aa, Mus musculus
ATFSLDS

SEQ ID NO: 6 - protein, 9 aa, Mus musculus
QQYANFPPT

SEQ ID NO: 7 - protein, 118 aa, Mus musculus
EVQLQQSGPELVKPGASVKMSCKASGYTFTNYVMHWVKQKPGQGLEWIGYFNPYNDGTNYNEKFKGKATLTSDKSSNTAYMELSSLTSEDSAVYYCARGGVRRYFDVWGAGTTVTVSS

SEQ ID NO: 8 - protein, 107 aa, Mus musculus
DIQMTQSPSSLSASLGERVSLTCRASQDIGSNLNWLQLGPDGTIKRLIYATFSLDSGVPKRFSGSRSGSDYSLTISSLESEDFVDYYCQQYANFPPTFGGGTKLEIK

SEQ ID NO: 9 - protein, 10 aa, Mus musculus
GFTFSNYGMS

SEQ ID NO: 10 - protein, 17 aa, Mus musculus
SISSGGGRIYYPDNVKG

SEQ ID NO: 11 - protein, 5 aa, Mus musculus
HAMDN

SEQ ID NO: 12 - protein, 10 aa, Mus musculus
SASSSVSNMY

SEQ ID NO: 13 - protein, 7 aa, Mus musculus
DTSKLAS

SEQ ID NO: 14 - protein, 9 aa, Mus musculus
QQWSSNPLT

SEQ ID NO: 15 - protein, 114 aa, Mus musculus
EVKLVESGGGLVKPGASLKLSCAASGFTFSNYGMSWVRQTSDKRLEWVASISSGGGRIYYPDNVKGRFTISRENAKNTLYLQMSSLKSEDTALYYCTRHAMDNWGQGTSVIVSS

SEQ ID NO: 16 - protein, 106 aa, Mus musculus
QIVLTQSPAIMSASPGEKVTMTCSASSSVSNMYWYQQKSGTSPKRWIYDTSKLASGVPARFSGSGSGTSYSLTISSMEAEDASTYYCQQWSSNPLTFGAGTTLELK

SEQ ID NO: 17 - protein, 10 aa, Mus musculus
GFTFSSYGMS

SEQ ID NO: 18 - protein, 17 aa, Mus musculus
TISSGGSYTYYPDSVKG

SEQ ID NO: 19 - protein, 9 aa, Mus musculus
QALRYHMDS

SEQ ID NO: 20 - protein, 11 aa, Mus musculus
KASQNVGTNVA

SEQ ID NO: 21 - protein, 7 aa, Mus musculus
SASYRYS

SEQ ID NO: 22 - protein, 9 aa, Mus musculus
QQYYSYPWT

SEQ ID NO: 23 - protein, 118 aa, Mus musculus
EVQLVESGGDLVKPGGSLKLSCAASGFTFSSYGMSWVRQTPDKRLEWVATISSGGSYTYYPDSVKGRFTFSRDNAKNTLYLQMSSLKSEDTAMYYCVRQALRYHMDSWGQGTSVTVSS

SEQ ID NO: 24 - protein, 107 aa, Mus musculus
DIVMTQSQKFMSTSVGDRVSVTCKASQNVGTNVAWYQQKPGQSPKALIYSASYRYSGVPDRFTGSGSGTDFTLTISNVQSEDLADFFCQQYYSYPWTFGGGTKLEIK

SEQ ID NO: 25 - protein, 10 aa, Mus musculus
GYTFTDYYMN

SEQ ID NO: 26 - protein, 17 aa, Mus musculus
YIYPNNGGTGYNQRFKG

SEQ ID NO: 27 - protein, 13 aa, Mus musculus
WGGTRLGYYAMDY

SEQ ID NO: 28 - protein, 11 aa, Mus musculus
KASQNVGTNVV

SEQ ID NO: 29 - protein, 7 aa, Mus musculus
WASTRHT

SEQ ID NO: 30 - protein, 9 aa, Mus musculus
QQYSRYPYT

SEQ ID NO: 31 - protein, 122 aa, Mus musculus
EVQLQQSGPELVKPGASVKMSCKASGYTFTDYYMNWVKQSHGKSLEWIGYIYPNNGGTGYNQRFKGKATLTADKSSSTAYMELRSLTSEDSAVYYCARWGGTRLGYYAMDYWGQGTSVTVSS

SEQ ID NO: 32 - protein, 107 aa, Mus musculus
DIVMTQSQKFMSTSVGDRVSVTCKASQNVGTNVVWYQQKPGQSPKLLIYWASTRHTGVPDRFTGSGSGTDFTLTISNVQSEDLADYFCQQYSRYPYTFGGGTKLEIK

SEQ ID NO: 33 - protein, 10 aa, Mus musculus
GFTFSSFGMH

SEQ ID NO: 34 - protein, 17 aa, Mus musculus
YISRGSSTIYYADTVKG

SEQ ID NO: 35 - protein, 12 aa, Mus musculus
SGYGSSSYYFDY

SEQ ID NO: 36 - protein, 12 aa, Mus musculus
RASSSIRSSYLH

SEQ ID NO: 37 - protein, 7 aa, Mus musculus
STSNLAS

SEQ ID NO: 38 - protein, 9 aa, Mus musculus
QQFSGYPLT

SEQ ID NO: 39 - protein, 121 aa, Mus musculus
DVQLVESGGGLVQPGGSRKVSCAASGFTFSSFGMHWVRQAPEKGLEWVAYISRGSSTIYYADTVKGRFTISRDNPKNTLFLQMTSLRSEDTAMYYCARSGYGSSSYYFDYWGQGTTLTVSS

SEQ ID NO: 40 - protein, 108 aa, Mus musculus
ENVLTQSPAIMSASPREKVTMTCRASSSIRSSYLHWYQQKSGASPKLWIYSTSNLASGVPARFSGSGSGTSYSLTISSVEAEDAATYYCQQFSGYPLTFGGGTKLEIK

SEQ ID NO: 41 - protein, 345 aa, Homo sapiens
MYKDCIESTGDYFLLCDAEGPWGIILESLAILGIVVTILLLLAFLFLMRKIQDCSQWNVLPTQLLFLLSVLGLFGLAFAFIIELNQQTAPVRYFLFGVLFALCFSCLLAHASNLVKLVRGCVSFSWTTILCIAIGCSLLQIIIATEYVTLIMTRGMMFVNMTPCQLNVDFVVLLVYVLFLMALTFFVSKATFCGPCENWKQHGRLIFITVLFSIIIWVVWISMLLRGNPQFQRQPQWDDPVVCIALVTNAWVFLLLYIVPELCILYRSCRQECPLQGNACPVTAYQHSFQVENQELSRARDSDGAEEDVALTSYGTPIQPQTVDPTQECFIPQAKLSPQQDAGGV

SEQ ID NO: 42 - protein, 344 aa, Macaca fascicularis
MYKDCIESTGDYFLPCDSEGPWGIILESLAILGIVVTILLLLAFLFLMRKIQDCSQWNVLPTQLLFLLSVLGLFGLAFAFIIQLNQQTAPVRYFLFGVLFALCFSCLLAHASNLVKLVRGRVSFSWTTILCIAIGCSLLQVIIAIEYVTLIMTRGMMFVHMTPYQLNVDFVVLLVYVLFLMALTFFVSKATFCGPCENWKQHGRLIFITVLFSIIIWVVWISMLLRGNPQFQRQPQWDDPVVCIALVTNAWVFLLLYIVPELCILYRSCRQECPSQGHACPVTAYQRSFQVENQELSRARDSDGAEEDVALTSFGTPIQPQTVDPTQECFIPRAKLSPQQDAGV

SEQ ID NO: 43 - protein, 344 aa, Mus musculus
MYEDCVKSTEDYYLFCDNEGPWAIVLESLAVIGIVVTILLLLAFLFLMRKVQDCSQWNVLPTQFLFLLAVLGLFGLTFAFIIQLNHQTAPVRYFLFGVLFAICFSCLLAHASNLVKLVRGRVSFCWTTILFIAIGVSLLQTIIAIEYVTLIMTRGLMFEHMTPYQLNVDFVCLLIYVLFLMALTFFVSKATFCGPCENWKQHGRLIFATVLVSIIIWVVWISMLLRGNPQLQRQPHWDDAVICIGLVTNAWVFLLIYIIPELSILYRSCRQECPTQGNVCQVPVYQRSFRMDTQEPTRARDSDGAQEDVALTAYGTPIQLQSADPSREYLIPSATLSPQQDAGL

SEQ ID NO: 44 - protein, 118 aa, synthetic construct
  REGION 1..118: note = VH of GC5B596; note (original language) = GC5B596的VH
QVQLVQSGAEVKKPGASVKVSCKASGYSFTGYTMNWVRQAPGQGLEWMGLINPYNSDTNYAQKLQGRVTMTTDTSTSTAYMELRSLRSDDTAVYYCARVALRVALDYWGQGTLVTVSS

SEQ ID NO: 45 - protein, 107 aa, synthetic construct
  REGION 1..107: note = VL of GC5B596; note (original language) = GC5B596的VL
DIQMTQSPSSLSASVGDRVTITCKASQNVATHVGWYQQKPGKAPKRLIYSASYRYSGVPSRFSGSGSGTEFTLTISNLQPEDFATYYCQQYNRYPYTFGQGTKLEIK

SEQ ID NO: 46 - protein, 357 aa, Homo sapiens
MATTVPDGCRNGLKSKYYRLCDKAEAWGIVLETVATAGVVTSVAFMLTLPILVCKVQDSNRRKMLPTQFLFLLGVLGIFGLTFAFIIGLDGSTGPTRFFLFGILFSICFSCLLAHAVSLTKLVRGRKPLSLLVILGLAVGFSLVQDVIAIEYIVLTMNRTNVNVFSELSAPRRNEDFVLLLTYVLFLMALTFLMSSFTFCGSFTGWKRHGAHIYLTMLLSIAIWVAWITLLMLPDFDRRWDDTILSSALAANGWVFLLAYVSPEFWLLTKQRNPMDYPVEDAFCKPQLVKKSYGVENRAYSQEEITQGFEETGDTLYAPYSTHFQLQNQPPQKEFSIPRAHAWPSPYKDYEVKKEGS

SEQ ID NO: 47 - protein, 403 aa, Homo sapiens
MFVASERKMRAHQVLTFLLLFVITSVASENASTSRGCGLDLLPQYVSLCDLDAIWGIVVEAVAGAGALITLLLMLILLVRLPFIKEKEKKSPVGLHFLFLLGTLGLFGLTFAFIIQEDETICSVRRFLWGVLFALCFSCLLSQAWRVRRLVRHGTGPAGWQLVGLALCLMLVQVIIAVEWLVLTVLRDTRPACAYEPMDFVMALIYDMVLLVVTLGLALFTLCGKFKRWKLNGAFLLITAFLSVLIWVAWMTMYLFGNVKLQQGDAWNDPTLAITLAASGWVFVIFHAIPEIHCTLLPALQENTPNYFDTSQPRMRETAFEEDVQLPRAYMENKAFSMDEHNAALRTAGFPNGSLGKRPSGSLGKRPSAPFRSNVYQPTEMAVVLNGGTIPTAPPSHTGRHLW

SEQ ID NO: 48 - protein, 441 aa, Homo sapiens
MAIHKALVMCLGLPLFLFPGAWAQGHVPPGCSQGLNPLYYNLCDRSGAWGIVLEAVAGAGIVTTFVLTIILVASLPFVQDTKKRSLLGTQVFFLLGTLGLFCLVFACVVKPDFSTCASRRFLFGVLFAICFSCLAAHVFALNFLARKNHGPRGWVIFTVALLLTLVEVIINTEWLIITLVRGSGEGGPQGNSSAGWAVASPCAIANMDFVMALIYVMLLLLGAFLGAWPALCGRYKRWRKHGVFVLLTTATSVAIWVVWIVMYTYGNKQHNSPTWDDPTLAIALAANAWAFVLFYVIPEVSQVTKSSPEQSYQGDMYPTRGVGYETILKEQKGQSMFVENKAFSMDEPVAAKRPVSPYSGYNGQLLTSVYQPTEMALMHKVPSEGAYDIILPRATANSQVMGSANSTLRAEDMYSAQSHQAATPPKDGKNSQVFRNPYVWD

SEQ ID NO: 49 - protein, 448 aa, synthetic construct
  REGION 1..448: note = Heavy chain of Chi-89; note (original language) = Chi-89的重链
EVQLVESGGDLVKPGGSLKLSCAASGFTFSSYGMSWVRQTPDKRLEWVATISSGGSYTYYPDSVKGRFTFSRDNAKNTLYLQMSSLKSEDTAMYYCVRQALRYHMDSWGQGTSVTVSSASTKGPSVFPLAPSSKSTSGGTAALGCLVKDYFPEPVTVSWNSGALTSGVHTFPAVLQSSGLYSLSSVVTVPSSSLGTQTYICNVNHKPSNTKVDKKVEPKSCDKTHTCPPCPAPELLGGPSVFLFPPKPKDTLMISRTPEVTCVVVDVSHEDPEVKFNWYVDGVEVHNAKTKPREEQYNSTYRVVSVLTVLHQDWLNGKEYKCKVSNKALPAPIEKTISKAKGQPREPQVYTLPPSRDELTKNQVSLTCLVKGFYPSDIAVEWESNGQPENNYKTTPPVLDSDGSFFLYSKLTVDKSRWQQGNVFSCSVMHEALHNHYTQKSLSLSPGK

SEQ ID NO: 50 - DNA, 1344 bp, synthetic construct
  source 1..1344: mol_type = other DNA
  gene 1..1344: note = Heavy chain of Chi-89; note (original language) = Chi-89的重链
gaggtgcagctggtggagtccggcggcgatctggtgaagcctggcggctccctgaagctgtcctgcgccgcttccggcttcaccttctcctcctacggcatgagctgggtgcggcagacccccgataagcggctggagtgggtggctaccatcagctccggcggcagctacacctactaccccgacagcgtgaagggccggttcaccttcagcagggataacgccaagaataccctgtatctgcagatgtccagcctgaagtccgaggacaccgccatgtattactgtgtgaggcaggctctgcggtaccacatggattcctggggccagggcacctccgtgaccgtgagcagcgcttctacaaagggaccttcagtgttccctctggctccgtcttcaaagagcactagcgggggaacagctgcactgggatgcctggtgaaggattacttccctgaacctgtgacagtgtcttggaacagcggggcattgactagtggagtccatacctttcctgcagtcctgcagtcttctggcctgtattcactgtcaagcgtggtgaccgtgcccagttcttccctgggtacccagacctatatttgcaatgtgaatcataagccaagcaataccaaggtcgacaaaaaggtggagcccaagagttgtgataagacccatacctgcccaccatgtccagcaccagagctgttggggggaccctctgtattcttgttcccacctaaacccaaggacacccttatgatctcacgcacccccgaagtcacatgtgttgtcgttgacgttagtcatgaggaccccgaggtcaagttcaattggtatgtcgacggcgtggaggtgcacaatgctaaaaccaaacctagagaagagcagtacaacagcacctacagagtggtctccgtgctgaccgttcttcaccaggattggttgaacggaaaagagtacaaatgcaaggttagcaacaaggcactgcccgctcctatcgaaaaaaccattagtaaagctaagggccagcctagagaaccgcaagtctataccttgccaccgtcacgagatgagctgaccaagaatcaagtgagcctgacttgcctggtcaagggattttacccatccgacatagctgtcgagtgggagtccaatggccagcccgaaaacaattacaagaccacacccccggtcctggattcagatggatcattcttcttgtactccaaacttacagtcgataaaagtcggtggcagcagggcaacgtgttctcctgctcagtgatgcacgaggccctgcataaccactacactcagaagtccctttccctttccccgggtaag

SEQ ID NO: 51 - protein, 214 aa, synthetic construct
  REGION 1..214: note = Light chain of Chi-89; note (original language) = Chi-89的轻链
DIVMTQSQKFMSTSVGDRVSVTCKASQNVGTNVAWYQQKPGQSPKALIYSASYRYSGVPDRFTGSGSGTDFTLTISNVQSEDLADFFCQQYYSYPWTFGGGTKLEIKRTVAAPSVFIFPPSDEQLKSGTASVVCLLNNFYPREAKVQWKVDNALQSGNSQESVTEQDSKDSTYSLSSTLTLSKADYEKHKVYACEVTHQGLSSPVTKSFNRGEC

SEQ ID NO: 52 - DNA, 642 bp, synthetic construct
  source 1..642: mol_type = other DNA
  gene 1..642: note = Light chain of Chi-89; note (original language) = Chi-89的轻链
gacatcgtgatgacccagagccagaagttcatgagcaccagcgtgggcgaccgggtgtccgtgacctgtaaggcttcccagaacgtgggcaccaacgtggcttggtaccagcagaagcctggccagagccccaaggccctgatctacagcgcctcctatcggtacagcggcgtgcctgacaggttcaccggctccggcagcggcaccgacttcaccctgaccatctccaacgtgcagagcgaggatctggccgacttcttctgtcagcagtactatagctacccttggaccttcggcggcggcaccaagctggagatcaagagaaccgtagccgctccaagtgtgtttattttccctccctcagacgagcagctgaagtccggcacagcatccgtagtgtgcctcttgaacaatttttaccctcgcgaggccaaggtgcagtggaaggtggataacgccctgcagagtggcaacagtcaggaatctgtgactgaacaggactccaaggactcaacctactcactgagctccaccctgacactgtctaaagctgattacgagaagcacaaggtatacgcttgcgaggtcacccatcaagggctgagcagccctgtgacaaaaagctttaacagaggcgagtgc

SEQ ID NO: 53 - protein, 452 aa, synthetic construct
  REGION 1..452: note = Heavy chain of Chi-105; note (original language) = Chi-105的重链
EVQLQQSGPELVKPGASVKMSCKASGYTFTDYYMNWVKQSHGKSLEWIGYIYPNNGGTGYNQRFKGKATLTADKSSSTAYMELRSLTSEDSAVYYCARWGGTRLGYYAMDYWGQGTSVTVSSASTKGPSVFPLAPSSKSTSGGTAALGCLVKDYFPEPVTVSWNSGALTSGVHTFPAVLQSSGLYSLSSVVTVPSSSLGTQTYICNVNHKPSNTKVDKKVEPKSCDKTHTCPPCPAPELLGGPSVFLFPPKPKDTLMISRTPEVTCVVVDVSHEDPEVKFNWYVDGVEVHNAKTKPREEQYNSTYRVVSVLTVLHQDWLNGKEYKCKVSNKALPAPIEKTISKAKGQPREPQVYTLPPSRDELTKNQVSLTCLVKGFYPSDIAVEWESNGQPENNYKTTPPVLDSDGSFFLYSKLTVDKSRWQQGNVFSCSVMHEALHNHYTQKSLSLSPGK

SEQ ID NO: 54 - DNA, 1356 bp, synthetic construct
  source 1..1356: mol_type = other DNA
  gene 1..1356: note = Heavy chain of Chi-105; note (original language) = Chi-105的重链
gaggtgcagctgcagcagagcggccccgagctggtgaagcccggagcttccgtgaagatgagctgcaaggcctccggctataccttcaccgactattacatgaactgggtgaagcagtcccacggcaagagcctggagtggatcggctatatctatcccaataacggcggcaccggctataatcagcggtttaagggcaaggctaccctgaccgccgacaagtcctccagcaccgcctatatggagctgcggagcctgacctccgaggatagcgccgtgtactactgtgctaggtggggcggcacccggctgggatactacgccatggattactggggccagggcacctccgtgaccgtgagcagcgcttctacaaagggaccttcagtgttccctctggctccgtcttcaaagagcactagcgggggaacagctgcactgggatgcctggtgaaggattacttccctgaacctgtgacagtgtcttggaacagcggggcattgactagtggagtccatacctttcctgcagtcctgcagtcttctggcctgtattcactgtcaagcgtggtgaccgtgcccagttcttccctgggtacccagacctatatttgcaatgtgaatcataagccaagcaataccaaggtcgacaaaaaggtggagcccaagagttgtgataagacccatacctgcccaccatgtccagcaccagagctgttggggggaccctctgtattcttgttcccacctaaacccaaggacacccttatgatctcacgcacccccgaagtcacatgtgttgtcgttgacgttagtcatgaggaccccgaggtcaagttcaattggtatgtcgacggcgtggaggtgcacaatgctaaaaccaaacctagagaagagcagtacaacagcacctacagagtggtctccgtgctgaccgttcttcaccaggattggttgaacggaaaagagtacaaatgcaaggttagcaacaaggcactgcccgctcctatcgaaaaaaccattagtaaagctaagggccagcctagagaaccgcaagtctataccttgccaccgtcacgagatgagctgaccaagaatcaagtgagcctgacttgcctggtcaagggattttacccatccgacatagctgtcgagtgggagtccaatggccagcccgaaaacaattacaagaccacacccccggtcctggattcagatggatcattcttcttgtactccaaacttacagtcgataaaagtcggtggcagcagggcaacgtgttctcctgctcagtgatgcacgaggccctgcataaccactacactcagaagtccctttccctttccccgggtaag

SEQ ID NO: 55 - protein, 214 aa, synthetic construct
  REGION 1..214: note = Light chain of Chi-105; note (original language) = Chi-105的轻链
DIVMTQSQKFMSTSVGDRVSVTCKASQNVGTNVVWYQQKPGQSPKLLIYWASTRHTGVPDRFTGSGSGTDFTLTISNVQSEDLADYFCQQYSRYPYTFGGGTKLEIKRTVAAPSVFIFPPSDEQLKSGTASVVCLLNNFYPREAKVQWKVDNALQSGNSQESVTEQDSKDSTYSLSSTLTLSKADYEKHKVYACEVTHQGLSSPVTKSFNRGEC

SEQ ID NO: 56 - DNA, 642 bp, synthetic construct
  source 1..642: mol_type = other DNA
  gene 1..642: note = Light chain of Chi-105; note (original language) = Chi-105的轻链
gatatcgtgatgacccagagccagaagttcatgagcaccagcgtgggcgaccgggtgagcgtgacctgcaaggccagccagaatgtgggcaccaacgtggtgtggtaccagcagaagcctggccagtcccctaagctgctgatctattgggccagcaccaggcacaccggcgtgccagaccggttcaccggctccggaagcggcaccgacttcaccctgaccatcagcaacgtgcagagcgaggacctggctgattacttctgccagcagtactccaggtatccctatacctttggcggcggcaccaagctggagatcaagagaaccgtagccgctccaagtgtgtttattttccctccctcagacgagcagctgaagtccggcacagcatccgtagtgtgcctcttgaacaatttttaccctcgcgaggccaaggtgcagtggaaggtggataacgccctgcagagtggcaacagtcaggaatctgtgactgaacaggactccaaggactcaacctactcactgagctccaccctgacactgtctaaagctgattacgagaagcacaaggtatacgcttgcgaggtcacccatcaagggctgagcagccctgtgacaaaaagctttaacagaggcgagtgc

SEQ ID NO: 57 - protein, 451 aa, synthetic construct
  REGION 1..451: note = Heavy chain of Chi-128; note (original language) = Chi-128的重链
DVQLVESGGGLVQPGGSRKVSCAASGFTFSSFGMHWVRQAPEKGLEWVAYISRGSSTIYYADTVKGRFTISRDNPKNTLFLQMTSLRSEDTAMYYCARSGYGSSSYYFDYWGQGTTLTVSASTKGPSVFPLAPSSKSTSGGTAALGCLVKDYFPEPVTVSWNSGALTSGVHTFPAVLQSSGLYSLSSVVTVPSSSLGTQTYICNVNHKPSNTKVDKKVEPKSCDKTHTCPPCPAPELLGGPSVFLFPPKPKDTLMISRTPEVTCVVVDVSHEDPEVKFNWYVDGVEVHNAKTKPREEQYNSTYRVVSVLTVLHQDWLNGKEYKCKVSNKALPAPIEKTISKAKGQPREPQVYTLPPSRDELTKNQVSLTCLVKGFYPSDIAVEWESNGQPENNYKTTPPVLDSDGSFFLYSKLTVDKSRWQQGNVFSCSVMHEALHNHYTQKSLSLSPGKS

SEQ ID NO: 58 - DNA, 1353 bp, synthetic construct
  source 1..1353: mol_type = other DNA
  gene 1..1353: note = Heavy chain of Chi-128; note (original language) = Chi-128的重链
gacgtgcagctggtggagagcggcggcggactggtgcagccaggaggatctcggaaggtgtcctgtgctgccagcggcttcaccttcagcagcttcggcatgcactgggtgaggcaggctcctgagaagggcctggagtgggtggcttatatctcccggggctcctccaccatctactatgctgataccgtgaagggcaggttcaccatctcccgggacaatcctaagaacaccctgttcctgcagatgacctccctgaggtccgaggacaccgctatgtattattgtgccaggtccggctatggctcctccagctattacttcgactactggggccagggcaccaccctgaccgtgtccagcgcttctacaaagggaccttcagtgttccctctggctccgtcttcaaagagcactagcgggggaacagctgcactgggatgcctggtgaaggattacttccctgaacctgtgacagtgtcttggaacagcggggcattgactagtggagtccatacctttcctgcagtcctgcagtcttctggcctgtattcactgtcaagcgtggtgaccgtgcccagttcttccctgggtacccagacctatatttgcaatgtgaatcataagccaagcaataccaaggtcgacaaaaaggtggagcccaagagttgtgataagacccatacctgcccaccatgtccagcaccagagctgttggggggaccctctgtattcttgttcccacctaaacccaaggacacccttatgatctcacgcacccccgaagtcacatgtgttgtcgttgacgttagtcatgaggaccccgaggtcaagttcaattggtatgtcgacggcgtggaggtgcacaatgctaaaaccaaacctagagaagagcagtacaacagcacctacagagtggtctccgtgctgaccgttcttcaccaggattggttgaacggaaaagagtacaaatgcaaggttagcaacaaggcactgcccgctcctatcgaaaaaaccattagtaaagctaagggccagcctagagaaccgcaagtctataccttgccaccgtcacgagatgagctgaccaagaatcaagtgagcctgacttgcctggtcaagggattttacccatccgacatagctgtcgagtgggagtccaatggccagcccgaaaacaattacaagaccacacccccggtcctggattcagatggatcattcttcttgtactccaaacttacagtcgataaaagtcggtggcagcagggcaacgtgttctcctgctcagtgatgcacgaggccctgcataaccactacactcagaagtccctttccctttccccgggtaag

SEQ ID NO: 59 - protein, 215 aa, synthetic construct
  REGION 1..215: note = Light chain of Chi-128; note (original language) = Chi-128的轻链
ENVLTQSPAIMSASPREKVTMTCRASSSIRSSYLHWYQQKSGASPKLWIYSTSNLASGVPARFSGSGSGTSYSLTISSVEAEDAATYYCQQFSGYPLTFGGGTKLEIKRTVAAPSVFIFPPSDEQLKSGTASVVCLLNNFYPREAKVQWKVDNALQSGNSQESVTEQDSKDSTYSLSSTLTLSKADYEKHKVYACEVTHQGLSSPVTKSFNRGEC

SEQ ID NO: 60 - DNA, 645 bp, synthetic construct
  source 1..645: mol_type = other DNA
  gene 1..645: note = Light chain of Chi-128; note (original language) = Chi-128的轻链
gagaacgtgctgacccagagccctgccatcatgagcgccagccctcgggagaaggtgaccatgacctgccgggcctcctcctccatcaggagcagctacctgcactggtaccagcagaagagcggcgccagccctaagctgtggatctactccacctccaatctggcctccggcgtgcccgccagattctccggaagcggcagcggcaccagctactccctgaccatcagctccgtggaggctgaggacgccgccacctattactgtcagcagttcagcggctaccctctgaccttcggcggcggcaccaagctggagatcaagagaaccgtagccgctccaagtgtgtttattttccctccctcagacgagcagctgaagtccggcacagcatccgtagtgtgcctcttgaacaatttttaccctcgcgaggccaaggtgcagtggaaggtggataacgccctgcagagtggcaacagtcaggaatctgtgactgaacaggactccaaggactcaacctactcactgagctccaccctgacactgtctaaagctgattacgagaagcacaaggtatacgcttgcgaggtcacccatcaagggctgagcagccctgtgacaaaaagctttaacagaggcgagtgc

SEQ ID NO: 61 - protein, 448 aa, synthetic construct
  REGION 1..448: note = Heavy chain of Chi-131; note (original language) = Chi-131的重链
EVQLQQSGPELVKPGASVKMSCKASGYTFTNYVMHWVKQKPGQGLEWIGYFNPYNDGTNYNEKFKGKATLTSDKSSNTAYMELSSLTSEDSAVYYCARGGVRRYFDVWGAGTTVTVSSASTKGPSVFPLAPSSKSTSGGTAALGCLVKDYFPEPVTVSWNSGALTSGVHTFPAVLQSSGLYSLSSVVTVPSSSLGTQTYICNVNHKPSNTKVDKKVEPKSCDKTHTCPPCPAPELLGGPSVFLFPPKPKDTLMISRTPEVTCVVVDVSHEDPEVKFNWYVDGVEVHNAKTKPREEQYNSTYRVVSVLTVLHQDWLNGKEYKCKVSNKALPAPIEKTISKAKGQPREPQVYTLPPSRDELTKNQVSLTCLVKGFYPSDIAVEWESNGQPENNYKTTPPVLDSDGSFFLYSKLTVDKSRWQQGNVFSCSVMHEALHNHYTQKSLSLSPGK

SEQ ID NO: 62 - DNA, 1344 bp, synthetic construct
  source 1..1344: mol_type = other DNA
  gene 1..1344: note = Heavy chain of Chi-131; note (original language) = Chi-131的重链
gaggtgcagctgcagcagtccggccccgagctggtgaagcctggcgctagcgtgaagatgtcctgcaaggcttccggctataccttcaccaattatgtgatgcactgggtgaagcagaagcccggccagggcctggagtggatcggctacttcaacccctacaatgatggcaccaactacaacgagaagttcaagggcaaggctaccctgaccagcgacaagtccagcaataccgcctatatggagctgagctccctgacctccgaggacagcgccgtgtattattgcgcccggggcggcgtgaggaggtacttcgatgtgtggggcgctggcaccaccgtgaccgtgtccagcgcttctacaaagggaccttcagtgttccctctggctccgtcttcaaagagcactagcgggggaacagctgcactgggatgcctggtgaaggattacttccctgaacctgtgacagtgtcttggaacagcggggcattgactagtggagtccatacctttcctgcagtcctgcagtcttctggcctgtattcactgtcaagcgtggtgaccgtgcccagttcttccctgggtacccagacctatatttgcaatgtgaatcataagccaagcaataccaaggtcgacaaaaaggtggagcccaagagttgtgataagacccatacctgcccaccatgtccagcaccagagctgttggggggaccctctgtattcttgttcccacctaaacccaaggacacccttatgatctcacgcacccccgaagtcacatgtgttgtcgttgacgttagtcatgaggaccccgaggtcaagttcaattggtatgtcgacggcgtggaggtgcacaatgctaaaaccaaacctagagaagagcagtacaacagcacctacagagtggtctccgtgctgaccgttcttcaccaggattggttgaacggaaaagagtacaaatgcaaggttagcaacaaggcactgcccgctcctatcgaaaaaaccattagtaaagctaagggccagcctagagaaccgcaagtctataccttgccaccgtcacgagatgagctgaccaagaatcaagtgagcctgacttgcctggtcaagggattttacccatccgacatagctgtcgagtgggagtccaatggccagcccgaaaacaattacaagaccacacccccggtcctggattcagatggatcattcttcttgtactccaaacttacagtcgataaaagtcggtggcagcagggcaacgtgttctcctgctcagtgatgcacgaggccctgcataaccactacactcagaagtccctttccctttccccgggtaag

SEQ ID NO: 63 - protein, 214 aa, synthetic construct
  REGION 1..214: note = Light chain L of Chi-131; note (original language) = Chi-131的轻链
DIQMTQSPSSLSASLGERVSLTCRASQDIGSNLNWLQLGPDGTIKRLIYATFSLDSGVPKRFSGSRSGSDYSLTISSLESEDFVDYYCQQYANFPPTFGGGTKLEIKRTVAAPSVFIFPPSDEQLKSGTASVVCLLNNFYPREAKVQWKVDNALQSGNSQESVTEQDSKDSTYSLSSTLTLSKADYEKHKVYACEVTHQGLSSPVTKSFNRGEC

SEQ ID NO: 64 - DNA, 642 bp, synthetic construct
  source 1..642: mol_type = other DNA
  gene 1..642: note = Light chain L of Chi-131; note (original language) = Chi-131的轻链
gacatccagatgacccagagcccctccagcctgagcgcctccctgggagagagggtgtccctgacctgccgggccagccaggacatcggctccaatctgaattggctgcagctgggccctgacggcaccatcaagaggctgatctacgctaccttcagcctggatagcggcgtgcctaagcggttctccggctccaggagcggctccgactatagcctgaccatcagctccctggagtccgaggacttcgtggattattactgtcagcagtatgccaacttcccccctaccttcggcggcggcaccaagctggagatcaagagaaccgtagccgctccaagtgtgtttattttccctccctcagacgagcagctgaagtccggcacagcatccgtagtgtgcctcttgaacaatttttaccctcgcgaggccaaggtgcagtggaaggtggataacgccctgcagagtggcaacagtcaggaatctgtgactgaacaggactccaaggactcaacctactcactgagctccaccctgacactgtctaaagctgattacgagaagcacaaggtatacgcttgcgaggtcacccatcaagggctgagcagccctgtgacaaaaagctttaacagaggcgagtgc

SEQ ID NO: 65 - protein, 444 aa, synthetic construct
  REGION 1..444: note = Heavy chain of Chi-169; note (original language) = Chi-169的重链
EVKLVESGGGLVKPGASLKLSCAASGFTFSNYGMSWVRQTSDKRLEWVASISSGGGRIYYPDNVKGRFTISRENAKNTLYLQMSSLKSEDTALYYCTRHAMDNWGQGTSVIVSSASTKGPSVFPLAPSSKSTSGGTAALGCLVKDYFPEPVTVSWNSGALTSGVHTFPAVLQSSGLYSLSSVVTVPSSSLGTQTYICNVNHKPSNTKVDKKVEPKSCDKTHTCPPCPAPELLGGPSVFLFPPKPKDTLMISRTPEVTCVVVDVSHEDPEVKFNWYVDGVEVHNAKTKPREEQYNSTYRVVSVLTVLHQDWLNGKEYKCKVSNKALPAPIEKTISKAKGQPREPQVYTLPPSRDELTKNQVSLTCLVKGFYPSDIAVEWESNGQPENNYKTTPPVLDSDGSFFLYSKLTVDKSRWQQGNVFSCSVMHEALHNHYTQKSLSLSPGK

SEQ ID NO: 66 - DNA, 1332 bp, synthetic construct
  source 1..1332: mol_type = other DNA
  gene 1..1332: note = Heavy chain of Chi-169; note (original language) = Chi-169的重链
gaggtgaagctggtggagagcggcggcggcctggtgaagcctggagcttctctgaagctgtcctgtgctgccagcggcttcaccttcagcaactatggcatgtcctgggtgaggcagacctccgacaagcggctggagtgggtggccagcatcagcagcggcggcggaagaatctattatcccgacaacgtgaagggccggttcaccatctcccgggagaatgccaagaataccctgtacctgcagatgtcctccctgaagtccgaggacaccgccctgtattattgcacccggcacgctatggataattggggccagggcaccagcgtgatcgtgagcagcgcttctacaaagggaccttcagtgttccctctggctccgtcttcaaagagcactagcgggggaacagctgcactgggatgcctggtgaaggattacttccctgaacctgtgacagtgtcttggaacagcggggcattgactagtggagtccatacctttcctgcagtcctgcagtcttctggcctgtattcactgtcaagcgtggtgaccgtgcccagttcttccctgggtacccagacctatatttgcaatgtgaatcataagccaagcaataccaaggtcgacaaaaaggtggagcccaagagttgtgataagacccatacctgcccaccatgtccagcaccagagctgttggggggaccctctgtattcttgttcccacctaaacccaaggacacccttatgatctcacgcacccccgaagtcacatgtgttgtcgttgacgttagtcatgaggaccccgaggtcaagttcaattggtatgtcgacggcgtggaggtgcacaatgctaaaaccaaacctagagaagagcagtacaacagcacctacagagtggtctccgtgctgaccgttcttcaccaggattggttgaacggaaaagagtacaaatgcaaggttagcaacaaggcactgcccgctcctatcgaaaaaaccattagtaaagctaagggccagcctagagaaccgcaagtctataccttgccaccgtcacgagatgagctgaccaagaatcaagtgagcctgacttgcctggtcaagggattttacccatccgacatagctgtcgagtgggagtccaatggccagcccgaaaacaattacaagaccacacccccggtcctggattcagatggatcattcttcttgtactccaaacttacagtcgataaaagtcggtggcagcagggcaacgtgttctcctgctcagtgatgcacgaggccctgcataaccactacactcagaagtccctttccctttccccgggtaag

SEQ ID NO: 67 - protein, 213 aa, synthetic construct
  REGION 1..213: note = Light chain of Chi-169; note (original language) = Chi-169的轻链
QIVLTQSPAIMSASPGEKVTMTCSASSSVSNMYWYQQKSGTSPKRWIYDTSKLASGVPARFSGSGSGTSYSLTISSMEAEDASTYYCQQWSSNPLTFGAGTTLELKRTVAAPSVFIFPPSDEQLKSGTASVVCLLNNFYPREAKVQWKVDNALQSGNSQESVTEQDSKDSTYSLSSTLTLSKADYEKHKVYACEVTHQGLSSPVTKSFNRGEC

SEQ ID NO: 68 - DNA, 639 bp, synthetic construct
  source 1..639: mol_type = other DNA
  gene 1..639: note = Light chain of Chi-169; note (original language) = Chi-169的轻链
cagatcgtgctgacccagtcccctgccatcatgtccgcttctcccggcgagaaggtgaccatgacctgttccgcctccagcagcgtgagcaatatgtactggtatcagcagaagtccggcacctcccctaagcggtggatctacgacacctccaagctggccagcggcgtgcctgctaggttctccggcagcggctccggcaccagctattccctgaccatcagcagcatggaggctgaggatgcttccacctactattgtcagcagtggtccagcaaccccctgaccttcggcgctggcaccaccctggagctgaagagaaccgtagccgctccaagtgtgtttattttccctccctcagacgagcagctgaagtccggcacagcatccgtagtgtgcctcttgaacaatttttaccctcgcgaggccaaggtgcagtggaaggtggataacgccctgcagagtggcaacagtcaggaatctgtgactgaacaggactccaaggactcaacctactcactgagctccaccctgacactgtctaaagctgattacgagaagcacaaggtatacgcttgcgaggtcacccatcaagggctgagcagccctgtgacaaaaagctttaacagaggcgagtgc

SEQ ID NO: 69 - protein, 330 aa, Homo sapiens [sequence omitted]

SEQ ID NO: 70 - protein, 107 aa, Homo sapiens [sequence omitted]

SEQ ID NO: 71 - protein, 5 aa, Mus musculus
NYVMH